European Patent Specification EP 4 070 855 B1, published December 24, 2025. Title: B-cell antibody receptor and use thereof. Applicant: Kyoto Prefectural Public University corporation MEDINET Co., Ltd. The sequence listing filed with the application follows.

SEQUENCE LISTING (44 sequences)

SEQ ID NO: 1 - DNA, 1194 bp, Homo sapiens
  DNA encoding alpha-GAL full length protein
ctggacaatggattggcaaggacgcctaccatgggctggctgcactgggagcgcttcatgtgcaaccttgactgccaggaagagccagattcctgcatcagtgagaagctcttcatggagatggcagagctcatggtctcagaaggctggaaggatgcaggttatgagtacctctgcattgatgactgttggatggctccccaaagagattcagaaggcagacttcaggcagaccctcagcgctttcctcatgggattcgccagctagctaattatgttcacagcaaaggactgaagctagggatttatgcagatgttggaaataaaacctgcgcaggcttccctgggagttttggatactacgacattgatgcccagacctttgctgactggggagtagatctgctaaaatttgatggttgttactgtgacagtttggaaaatttggcagatggttataagcacatgtccttggccctgaataggactggcagaagcattgtgtactcctgtgagtggcctctttatatgtggccctttcaaaagcccaattatacagaaatccgacagtactgcaatcactggcgaaattttgctgacattgatgattcctggaaaagtataaagagtatcttggactggacatcttttaaccaggagagaattgttgatgttgctggaccagggggttggaatgacccagatatgttagtgattggcaactttggcctcagctggaatcagcaagtaactcagatggccctctgggctatcatggctgctcctttattcatgtctaatgacctccgacacatcagccctcaagccaaagctctccttcaggataaggacgtaattgccatcaatcaggaccccttgggcaagcaagggtaccagcttagacagggagacaactttgaagtgtgggaacgacctctctcaggcttagcctgggctgtagctatgataaaccggcaggagattggtggacctcgctcttataccatcgcagttgcttccctgggtaaaggagtggcctgtaatcctgcctgcttcatcacacagctcctccctgtgaaaaggaagctagggttctatgaatggacttcaaggttaagaagtcacataaatcccacaggcactgttttgcttcagctagaaaatacaatgcagatgtcattaaaagacttactt

SEQ ID NO: 2 - DNA, 897 bp, Homo sapiens
  DNA encoding alpha-GAL D1 region protein
ctggacaatggattggcaaggacgcctaccatgggctggctgcactgggagcgcttcatgtgcaaccttgactgccaggaagagccagattcctgcatcagtgagaagctcttcatggagatggcagagctcatggtctcagaaggctggaaggatgcaggttatgagtacctctgcattgatgactgttggatggctccccaaagagattcagaaggcagacttcaggcagaccctcagcgctttcctcatgggattcgccagctagctaattatgttcacagcaaaggactgaagctagggatttatgcagatgttggaaataaaacctgcgcaggcttccctgggagttttggatactacgacattgatgcccagacctttgctgactggggagtagatctgctaaaatttgatggttgttactgtgacagtttggaaaatttggcagatggttataagcacatgtccttggccctgaataggactggcagaagcattgtgtactcctgtgagtggcctctttatatgtggccctttcaaaagcccaattatacagaaatccgacagtactgcaatcactggcgaaattttgctgacattgatgattcctggaaaagtataaagagtatcttggactggacatcttttaaccaggagagaattgttgatgttgctggaccagggggttggaatgacccagatatgttagtgattggcaactttggcctcagctggaatcagcaagtaactcagatggccctctgggctatcatggctgctcctttattcatgtctaatgacctccgacacatcagccctcaagccaaagctctccttcaggataaggacgtaattgccatcaatcaggaccccttgggcaagcaagggtaccag

SEQ ID NO: 3 - DNA, 375 bp, Homo sapiens
  DNA encoding ADAMTS13 spacer domain
agcccacggaagggctctttcacagctggcagagcgagagaatatgtcacgtttctgacagttacccccaacctgaccagtgtctacattgccaaccacaggcctctcttcacacacttggcggtgaggatcggagggcgctatgtcgtggctgggaagatgagcatctcccctaacaccacctacccctccctcctggaggatggtcgtgtcgagtacagagtggccctcaccgaggaccggctgccccgcctggaggagatccgcatctggggacccctccaggaagatgctgacatccaggtttacaggcggtatggcgaggagtatggcaacctcacccgcccagacatcaccttcacctacttccagcct

SEQ ID NO: 4 - DNA, 348 bp, Homo sapiens
  DNA encoding ADAMTS13 cysteine rich domain
aagacccagctggagttcatgtcgcaacagtgcgccaggaccgacggccagccgctgcgctcctcccctggcggcgcctccttctaccactggggtgctgctgtaccacacagccaaggggatgctctgtgcagacacatgtgccgggccattggcgagagcttcatcatgaagcgtggagacagcttcctcgatgggacccggtgtatgccaagtggcccccgggaggacgggaccctgagcctgtgtgtgtcgggcagctgcaggacatttggctgtgatggtaggatggactcccagcaggtatgggacaggtgccaggtgtgtggtggggacaacagcacgtgc

SEQ ID NO: 5 - DNA, 93 bp, Homo sapiens
  DNA encoding Signal Sequence Leader2
atgcagctgaggaacccagaactacatctgggctgcgcgcttgcgcttcgcttcctggccctcgtttcctgggacatccctggggctagagca

SEQ ID NO: 6 - DNA, 72 bp, Homo sapiens
  DNA encoding Transmembrane Domain
atctacatctgggcgcccttggccgggacttgtggggtccttctcctgtcactggttatcaccctttactgc

SEQ ID NO: 7 - DNA, 126 bp, Homo sapiens
  DNA encoding 4-1BB
aaacggggcagaaagaaactcctgtatatattcaaacaaccatttatgagaccagtacaaactactcaagaggaagatggctgtagctgccgatttccagaagaagaagaaggaggatgtgaactg

SEQ ID NO: 8 - DNA, 336 bp, Homo sapiens
  DNA encoding CD3 zeta
agagtgaagttcagcaggagcgcagacgcccccgcgtacaagcagggccagaaccagctctataacgagctcaatctaggacgaagagaggagtacgatgttttggacaagagacgtggccgggaccctgagatggggggaaagccgagaaggaagaaccctcaggaaggcctgtacaatgaactgcagaaagataagatggcggaggcctacagtgagattgggatgaaaggcgagcgccggaggggcaaggggcacgatggcctttaccagggtctcagtacagccaccaaggacacctacgacgcccttcacatgcaggccctgccccctcgc

SEQ ID NO: 9 - DNA, 750 bp, Homo sapiens
  DNA encoding scFv_anti-GLA
gacattgtgatgtcacagtctccatcctccctggctgtgtcagcaggagagaaggtcactatgagctgcaaatccagtcagagtctgctcaacagtagaacccgaaagaactacttggcttggtaccagcagaaaccagggcagtctcctaaactgctgatctactgggcatccactagggaatctggggtccctgatcgcttcacaggcagtggatctgggacagatttcactctcaccatcaccagtgtgcaggctgaagacctggcagtttattactgcaagcaatcttataatctgtggacgttcggtggaggcaccaagctggaaatcaaaggtggcggcggtagcggaggcggtgggagtggcggaggtggtagtggcggcggcggtagccaggtgcagctgaaggagtcaggacctggcctggtggcgccctcacagagcctgtccatcacttgcactgtctctgggttttcattaactagctttggtgtacattgggttcgccagcctccaggaaagggtctggagtggctgggagtaatatgggctggtggaagcacacattataattcggctctcatgtccagactgagcatcagcaaagacaactccaagagccaagttttcttaaaaatgaacagtctgcaaactgatgacacagccatgtactactgtgccagagagaattactacggtagtagcgcggactactggggccaaggcaccactctcacagtctcctca

SEQ ID NO: 10 - protein, 398 aa, Homo sapiens
  GLA Full Length protein
LDNGLARTPTMGWLHWERFMCNLDCQEEPDSCISEKLFMEMAELMVSEGWKDAGYEYLCIDDCWMAPQRDSEGRLQADPQRFPHGIRQLANYVHSKGLKLGIYADVGNKTCAGFPGSFGYYDIDAQTFADWGVDLLKFDGCYCDSLENLADGYKHMSLALNRTGRSIVYSCEWPLYMWPFQKPNYTEIRQYCNHWRNFADIDDSWKSIKSILDWTSFNQERIVDVAGPGGWNDPDMLVIGNFGLSWNQQVTQMALWAIMAAPLFMSNDLRHISPQAKALLQDKDVIAINQDPLGKQGYQLRQGDNFEVWERPLSGLAWAVAMINRQEIGGPRSYTIAVASLGKGVACNPACFITQLLPVKRKLGFYEWTSRLRSHINPTGTVLLQLENTMQMSLKDLL

SEQ ID NO: 11 - protein, 299 aa, Homo sapiens
  GLA D1 Region protein
LDNGLARTPTMGWLHWERFMCNLDCQEEPDSCISEKLFMEMAELMVSEGWKDAGYEYLCIDDCWMAPQRDSEGRLQADPQRFPHGIRQLANYVHSKGLKLGIYADVGNKTCAGFPGSFGYYDIDAQTFADWGVDLLKFDGCYCDSLENLADGYKHMSLALNRTGRSIVYSCEWPLYMWPFQKPNYTEIRQYCNHWRNFADIDDSWKSIKSILDWTSFNQERIVDVAGPGGWNDPDMLVIGNFGLSWNQQVTQMALWAIMAAPLFMSNDLRHISPQAKALLQDKDVIAINQDPLGKQGYQ

SEQ ID NO: 12 - protein, 125 aa, Homo sapiens
  ADAMTS13 spacer domain protein
SPRKGSFTAGRAREYVTFLTVTPNLTSVYIANHRPLFTHLAVRIGGRYVVAGKMSISPNTTYPSLLEDGRVEYRVALTEDRLPRLEEIRIWGPLQEDADIQVYRRYGEEYGNLTRPDITFTYFQP

SEQ ID NO: 13 - protein, 116 aa, Homo sapiens
  ADAMTS13 cysteine rich domain
KTQLEFMSQQCARTDGQPLRSSPGGASFYHWGAAVPHSQGDALCRHMCRAIGESFIMKRGDSFLDGTRCMPSGPREDGTLSLCVSGSCRTFGCDGRMDSQQVWDRCQVCGGDNSTC

SEQ ID NO: 14 - protein, 31 aa, Homo sapiens
  Signal Sequence Leader2 protein
MQLRNPELHLGCALALRFLALVSWDIPGARA

SEQ ID NO: 15 - protein, 24 aa, Homo sapiens
  Transmembrane Domain protein
IYIWAPLAGTCGVLLLSLVITLYC

SEQ ID NO: 16 - protein, 42 aa, Homo sapiens
  4-1BB protein
KRGRKKLLYIFKQPFMRPVQTTQEEDGCSCRFPEEEEGGCEL

SEQ ID NO: 17 - protein, 112 aa, Homo sapiens
  CD3 zeta protein
RVKFSRSADAPAYKQGQNQLYNELNLGRREEYDVLDKRRGRDPEMGGKPRRKNPQEGLYNELQKDKMAEAYSEIGMKGERRRGKGHDGLYQGLSTATKDTYDALHMQALPPR

SEQ ID NO: 18 - protein, 250 aa, Homo sapiens
  scFv anti-GLA protein
DIVMSQSPSSLAVSAGEKVTMSCKSSQSLLNSRTRKNYLAWYQQKPGQSPKLLIYWASTRESGVPDRFTGSGSGTDFTLTITSVQAEDLAVYYCKQSYNLWTFGGGTKLEIKGGGGSGGGGSGGGGSGGGGSQVQLKESGPGLVAPSQSLSITCTVSGFSLTSFGVHWVRQPPGKGLEWLGVIWAGGSTHYNSALMSRLSISKDNSKSQVFLKMNSLQTDDTAMYYCARENYYGSSADYWGQGTTLTVSS

SEQ ID NO: 19 - DNA, 36 bp, Artificial Sequence
  Alpha-GAL primer (forward)
aattagatctctcgaggccaccatgcagctgaggaa

SEQ ID NO: 20 - DNA, 62 bp, Artificial Sequence
  Alpha-GAL primer (reverse: full length)
ccagatgtagatatcacaggcgctaccgccgccaccggatccaagtaagtcttttaatgaca

SEQ ID NO: 21 - DNA, 50 bp, Artificial Sequence
  Alpha-GAL primer (reverse: D1)
ccagatgtagatatcaccgccaccggatccctggtacccttgcttgccca

SEQ ID NO: 22 - DNA, 20 bp, Artificial Sequence
  TM, 4-1BB, CD3z primer (forward)
gatatctacatctgggcgcc

SEQ ID NO: 23 - DNA, 36 bp, Artificial Sequence
  TM, 4-1BB, CD3z primer (reverse)
ctacccggtagaattcttagcgagggggcagggcct

SEQ ID NO: 24 - DNA, 63 bp, Homo sapiens
  DNA encoding Signal sequence Leader1
atggccttaccagtgaccgccttgctcctgccgctggccttgctgctccacgccgccaggccg

SEQ ID NO: 25 - protein, 21 aa, Homo sapiens
  Signal sequence Leader1 protein
MALPVTALLLPLALLLHAARP

SEQ ID NO: 26 - DNA, 63 bp, Homo sapiens; identical to SEQ ID NO: 24
  DNA encoding human CD8 signal peptide

SEQ ID NO: 27 - protein, 21 aa, Homo sapiens
  Human CD8 signal peptide
MALPVTALLLPLALLLHAARP

SEQ ID NO: 28 - DNA, 27 bp, Artificial sequence
  DNA encoding HA
tacccatacgacgtaccagattacgct

SEQ ID NO: 29 - protein, 9 aa, Artificial sequence
  HA protein
YPYDVPDYA

SEQ ID NO: 30 - DNA, 63 bp, Homo sapiens
  DNA encoding IgG4 antibody, hinge region
gtggaatctaagtatggtcctccgtgccccagttgccctgcaccggagtttctcggtggcccg

SEQ ID NO: 31 - protein, 21 aa, Homo sapiens
  IgG4 antibody, hinge region protein
VESKYGPPCPSCPAPEFLGGP

SEQ ID NO: 32 - DNA, 66 bp, Homo sapiens
  DNA encoding human IgG anti GLA antibody light chain
atggacatgagggtccctgctcagctcctggggctcctgctgctctggctctcaggtgccagatgt

SEQ ID NO: 33 - protein, 22 aa, Homo sapiens
  Human IgG anti GLA antibody light chain protein
MDMRVPAQLLGLLLLWLSGARC

SEQ ID NO: 34 - DNA, 705 bp, Artificial Sequence
  DNA encoding mCherry
gtgagcaagggcgaggaggataacatggccatcatcaaggagttcatgcgcttcaaggtgcacatggagggctccgtgaacggccacgagttcgagatcgagggcgagggcgagggccgcccctacgagggcacccagaccgccaagctgaaggtgaccaagggtggccccctgcccttcgcctgggacatcctgtcccctcagttcatgtacggctccaaggcctacgtgaagcaccccgccgacatccccgactacttgaagctgtccttccccgagggcttcaagtgggagcgcgtgatgaacttcgaggacggcggcgtggtgaccgtgacccaggactcctccctgcaggacggcgagttcatctacaaggtgaagctgcgcggcaccaacttcccctccgacggccccgtaatgcagaagaagaccatgggctgggaggcctcctccgagcggatgtaccccgaggacggcgccctgaagggcgagatcaagcagaggctgaagctgaaggacggcggccactacgacgctgaggtcaagaccacctacaaggccaagaagcccgtgcagctgcccggcgcctacaacgtcaacatcaagttggacatcacctcccacaacgaggactacaccatcgtggaacagtacgaacgcgccgagggccgccactccaccggcggcatggacgagctgtacaag

SEQ ID NO: 35 - protein, 235 aa, Artificial Sequence
  mCherry Protein
VSKGEEDNMAIIKEFMRFKVHMEGSVNGHEFEIEGEGEGRPYEGTQTAKLKVTKGGPLPFAWDILSPQFMYGSKAYVKHPADIPDYLKLSFPEGFKWERVMNFEDGGVVTVTQDSSLQDGEFIYKVKLRGTNFPSDGPVMQKKTMGWEASSERMYPEDGALKGEIKQRLKLKDGGHYDAEVKTTYKAKKPVQLPGAYNVNIKLDITSHNEDYTIVEQYERAEGRHSTGGMDELYK

SEQ ID NO: 36 - DNA, 750 bp, Homo sapiens
  DNA encoding scFv of anti GLA antibody
gacatcgtgatgtcccagagcccgtcaagtttggcggtgagcgcaggggaaaaggtaaccatgtcatgtaagagctcccaaagtctcttgaattcaaggacgcgaaagaattacctcgcatggtatcagcagaagccggggcaatcaccgaagctcttgatttattgggcgagcactcgagaaagcggggtgcccgatcggttcaccgggagcggaagcggcacagactttacactgaccataacgtccgtccaggctgaggatctggctgtctattattgcaaacaatcctataatctctggacattcggcggtgggaccaagcttgaaataaagggcgggggcgggagtggaggtggtggttctggaggtggagggtcagggggagggggtagtcaagtacaactcaaagagtctggtcccgggcttgtcgctccgtctcagtccctctcaataacctgtacagtaagtggattttcccttacttccttcggggtgcattgggtacgccagccgccgggtaaaggattggaatggctcggcgttatctgggcgggtggttctacacattacaacagcgcccttatgtcccgcttgtccatcagcaaggataacagtaagagccaggtgttccttaaaatgaactccctccagacagatgacacagcgatgtactattgtgcaagagagaattattacggctccagtgccgattattgggggcaaggaaccacgttgaccgttagttca

SEQ ID NO: 37 - DNA, 390 bp, Homo sapiens
  DNA encoding ADAMTS13 spacer domain
agcccacggaagggctctttcacagctggcagagcgagagaatatgtcacgtttctgacagttacccccaacctgaccagtgtctacattgccaaccacaggcctctcttcacacacttggcggtgaggatcggagggcgctatgtcgtggctgggaagatgagcatctcccctaacaccacctacccctccctcctggaggatggtcgtgtcgagtacagagtggccctcaccgaggaccggctgccccgcctggaggagatccgcatctggggacccctccaggaagatgctgacatccaggtttacaggcggtatggcgaggagtatggcaacctcacccgcccagacatcaccttcacctacttccagcctaagccacggcaggcc

SEQ ID NO: 38 - protein, 130 aa, Homo sapiens
  ADAMTS13 spacer domain protein
SPRKGSFTAGRAREYVTFLTVTPNLTSVYIANHRPLFTHLAVRIGGRYVVAGKMSISPNTTYPSLLEDGRVEYRVALTEDRLPRLEEIRIWGPLQEDADIQVYRRYGEEYGNLTRPDITFTYFQPKPRQA

SEQ ID NO: 39 - DNA, 66 bp, Homo sapiens
  DNA encoding signal peptide of human IgG anti ADAMTS13 antibody light chain
atggacatgagggttcctgcacaactccttgggctgctcttgttgtggttgtctggagcgcggtgt

SEQ ID NO: 40 - protein, 22 aa, Homo sapiens
  Signal peptide of Human IgG anti ADAMTS13 antibody light chain
MDMRVPAQLLGLLLLWLSGARC

SEQ ID NO: 41 - DNA, 738 bp, Homo sapiens
  DNA encoding scFv of anti ADAMTS13 antibody
caagtacaactcgtgcagagcggggcagaagttaaaaagcctggcagctccgtaaaagtcagctgtaaggcatctggaggggcgttcactatgtacactataaactgggttagacaggcaccaggtagaggcttggaatggatgggtcggatcattccgatcttgggaattaccgattatgctcagaagtttcaggggaggggcaccattacagccgataagagtacctctacagcgtatttggaactgtctgggctgacctctgaggataccgctgtgtattgcgcaagggagtttagcggaggaaattacttcgatttttggggacagggcacactggtgacggttagcagtggaggtggagggagtggaggaggtggtagtggcggaggtggatccggtgggggagggtcagagcttgagttgacccaaccgccgtccgtgtcaatttctcctggtaaaactgcaaagatattttgcggtggcaatagtattgggcgaaagtctgttaattggtatcaacaaaaacctggccaggcaccagttctcgtcgtatatgacgactccgatcgaccgagtggcatacccgaaaggttcagcggtagcaatagtgggaacactgctacccttaccatctccagggttgaggcaggcgacgaagctgattattactgtcaggtttgggattcaagttccgattactgggtctttggaggtgggacgaagctcacagtattg

SEQ ID NO: 42 - protein, 246 aa, Homo sapiens
  scFv of anti ADAMTS13 antibody
QVQLVQSGAEVKKPGSSVKVSCKASGGAFTMYTINWVRQAPGRGLEWMGRIIPILGITDYAQKFQGRGTITADKSTSTAYLELSGLTSEDTAVYCAREFSGGNYFDFWGQGTLVTVSSGGGGSGGGGSGGGGSGGGGSELELTQPPSVSISPGKTAKIFCGGNSIGRKSVNWYQQKPGQAPVLVVYDDSDRPSGIPERFSGSNSGNTATLTISRVEAGDEADYYCQVWDSSSDYWVFGGGTKLTVL

SEQ ID NO: 43 - DNA, 72 bp, Homo sapiens; identical to SEQ ID NO: 6
  DNA encoding transmembrane domain of Human CD8a

SEQ ID NO: 44 - protein, 24 aa, Homo sapiens
  Transmembrane domain of Human CD8a
IYIWAPLAGTCGVLLLSLVITLYC